European Patent Application EP 4 212 532 A2, published July 19, 2023. Title: MITRAGYNINE ANALOGS AND USES THEREOF. Applicant: MEMORIAL SLOAN-KETTERING CANCER CENTER. Application EP, filed April 29, 2016. The sequence listing filed with the application follows.

SEQUENCE LISTING (5 sequences)

SEQ ID NO: 1 - DNA, 19 bp, synthetic construct
  source 1..19: mol_type = other DNA
  misc_feature 1..19: note = Synthetic Polynucleotide
cgccccagcctcttcctct

SEQ ID NO: 2 - DNA, 18 bp, synthetic construct
  source 1..18: mol_type = other DNA
  misc_feature 1..18: note = Synthetic Polynucleotide
aggggaaggtcgggtagg

SEQ ID NO: 3 - DNA, 19 bp, synthetic construct
  source 1..19: mol_type = other DNA
  misc_feature 1..19: note = Synthetic Polynucleotide
cgccccgacctcttccctt

SEQ ID NO: 4 - DNA, 18 bp, synthetic construct
  source 1..18: mol_type = other DNA
  misc_feature 1..18: note = Synthetic Polynucleotide
gaggagaggtgcgtggag

SEQ ID NO: 5 - DNA, 19 bp, synthetic construct
  misc_feature 1..19: note = Synthetic Polynucleotide
  source 1..19: mol_type = other DNA
ctccgcgctctcaccctct